European Patent Specification EP 3 762 489 B1, published July 19, 2023. Title: Methods and Compositions for Live Cell Analysis of Intracellular ATP. Applicant: Essen BioScience, Inc. d/b/a Essen BioScience, Inc. Appledorn, Daniel Schramm, Cicely Filonov, Grigory Schroeder, Kirk S. The sequence listing filed with the application follows.

SEQUENCE LISTING (22 sequences)

SEQ ID NO: 1 - protein, 218 aa, Artificial Sequence
  Synthetic
  MISC_FEATURE (1)..(5): optionally absent
  MISC_FEATURE (217)..(218): optionally absent
MVSVIKPEMKMRYYMDGSVNGHEFTIEGEGTGRPYEGHQEMTLRVTMAEGGPMPFAFDLVSHVFCYGHRVFTKYPEEIPDYFKQAFPEGLSWERSLEFEDGGSASVSAHISLRGNTFYHKSKFTGVNFPADGPIMQNQSVDWEPSTEKITASDGVLKGDVTMYLKLEGGGNHKCQFKTTYKAAKEILEMPGDHYIGHRLVRKTEGNITEQVEDAVAHS

SEQ ID NO: 2 - protein, 217 aa, Artificial Sequence
  Synthetic
  MISC_FEATURE (1)..(5): optionally absent
  MISC_FEATURE (216)..(217): optionally absent
MSVIKPEMKMRYYMDGSVNGHEFTIEGEGTGRPYEGHQEMTLRVTMAKGGPMPFAFDLVSHVFCYGHRPFTKYPEEIPDYFKQAFPEGLSWERSLEFEDGGSASVSAHISLRGNTFYHKSKFTGVNFPADGPIMQNQSVDWEPSTEKITASDGVLKGDVTMYLKLEGGGNHKCQFKTTYKAAKKILKMPGSHYISHRLVRKTEGNITELVEDAVAHS

SEQ ID NO: 3 - protein, 218 aa, Artificial Sequence
  Synthetic
  MISC_FEATURE (1)..(5): optionally absent
  MISC_FEATURE (217)..(218): optionally absent
MVSVIKPEMKMRYYMDGSVNGHEFTIEGEGTGRPYEGHQEMTLRVTMAEGGPMPFAFDLVSHVFCYGHRVFTKYPEEIPDYFKQAFPEGLSWERSLEFEDGGSASVSAHISLRGNTFYHKSKFTGVNFPADGPIMQNQSVDWEPSTEKITASDGVLKGDVTMYLKLEGGGNHKCQMKTTYKAAKEILEMPGDHYIGHRLVRKTEGNITEQVEDAVAHS

SEQ ID NO: 4 - protein, 246 aa, Artificial Sequence
  Synthetic
  MISC_FEATURE (1)..(2): optionally absent
  MISC_FEATURE (34)..(34): Xaa is A or K
  MISC_FEATURE (245)..(246): optionally absent
DGSVQLADHYQQNTPIGDGPVLLPDNHYLSTQSXLSKDPNEKRDHMVLLEFVTAAGITLGMDELYKGGSGGMVSKGEELFTGVVPILVELDGDVNGHKFSVSGEGEGDATYGKLTLKFICTTGKLPVPWPTLVTTLTYGVQCFSRYPDHMKQHDFFKSAMPEGYVQERTIFFKDDGNYKTRAEVKFEGDTLVNRIELKGIDFKEDGNILGHKLEYNYNSHNVYIMADKQKNGIKVNFKIRHNIEEA

SEQ ID NO: 5 - protein, 132 aa, Artificial Sequence
  Synthetic
  MISC_FEATURE (1)..(1): optionally absent
MKTVKVNITTPDGPVYDADIEMVSVRAESGDLGILPGHIPTKAPLKIGAVRLKKDGQTEMVAVSGGTVEVRPDHVTINAQAAETAEGIDKERAEAARQRAQERLNSQSDDTDIRRAELALQRALNRLDVAGK

SEQ ID NO: 6 - protein, 133 aa, Artificial Sequence
  Synthetic
  MISC_FEATURE (1)..(1): optionally absent
MKTVKVNITTPDGPVYDADIEMVSVRAESGDLGILPGHIPTKAPLKIGAVRLKKDGQTEYVAVSGGTVEVRPDHVTINAQAAETAEGIDKERAEAARQRAQERLNSQSDDTDIRRAELALQRALNRLDVAEMK

SEQ ID NO: 7 - protein, 598 aa, Artificial Sequence
  Synthetic
  MISC_FEATURE (1)..(1): optionally absent
  MISC_FEATURE (220)..(220): optionally absent
MVSVIKPEMKMRYYMDGSVNGHEFTIEGEGTGRPYEGHQEMTLRVTMAEGGPMPFAFDLVSHVFCYGHRVFTKYPEEIPDYFKQAFPEGLSWERSLEFEDGGSASVSAHISLRGNTFYHKSKFTGVNFPADGPIMQNQSVDWEPSTEKITASDGVLKGDVTMYLKLEGGGNHKCQFKTTYKAAKEILEMPGDHYIGHRLVRKTEGNITEQVEDAVAHSAMKTVKVNITTPDGPVYDADIEMVSVRAESGDLGILPGHIPTKAPLKIGAVRLKKDGQTEMVAVSGGTVEVRPDHVTINAQAAETAEGIDKERAEAARQRAQERLNSQSDDTDIRRAELALQRALNRLDVAGKADGSVQLADHYQQNTPIGDGPVLLPDNHYLSTQSKLSKDPNEKRDHMVLLEFVTAAGITLGMDELYKGGSGGMVSKGEELFTGVVPILVELDGDVNGHKFSVSGEGEGDATYGKLTLKFICTTGKLPVPWPTLVTTLTYGVQCFSRYPDHMKQHDFFKSAMPEGYVQERTIFFKDDGNYKTRAEVKFEGDTLVNRIELKGIDFKEDGNILGHKLEYNYNSHNVYIMADKQKNGIKVNFKIRHNIEEA

SEQ ID NO: 8 - protein, 598 aa, Artificial Sequence
  Synthetic
  MISC_FEATURE (1)..(1): optionally absent
  MISC_FEATURE (220)..(220): optionally absent
MVSVIKPEMKMRYYMDGSVNGHEFTIEGEGTGRPYEGHQEMTLRVTMAEGGPMPFAFDLVSHVFCYGHRVFTKYPEEIPDYFKQAFPEGLSWERSLEFEDGGSASVSAHISLRGNTFYHKSKFTGVNFPADGPIMQNQSVDWEPSTEKITASDGVLKGDVTMYLKLEGGGNHKCQFKTTYKAAKEILEMPGDHYIGHRLVRKTEGNITEQVEDAVAHSSMKTVKVNITTPDGPVYDADIEMVSVRAESGDLGILPGHIPTKAPLKIGAVRLKKDGQTEMVAVSGGTVEVRPDHVTINAQAAETAEGIDKERAEAARQRAQERLNSQSDDTDIRRAELALQRALNRLDVAGKADGSVQLADHYQQNTPIGDGPVLLPDNHYLSTQSKLSKDPNEKRDHMVLLEFVTAAGITLGMDELYKGGSGGMVSKGEELFTGVVPILVELDGDVNGHKFSVSGEGEGDATYGKLTLKFICTTGKLPVPWPTLVTTLTYGVQCFSRYPDHMKQHDFFKSAMPEGYVQERTIFFKDDGNYKTRAEVKFEGDTLVNRIELKGIDFKEDGNILGHKLEYNYNSHNVYIMADKQKNGIKVNFKIRHNIEEA

SEQ ID NO: 9 - protein, 598 aa, Artificial Sequence
  Synthetic
  MISC_FEATURE (1)..(1): optionally absent
  MISC_FEATURE (219)..(219): optionally absent
MVSVIKPEMKMRYYMDGSVNGHEFTIEGEGTGRPYEGHQEMTLRVTMAEGGPMPFAFDLVSHVFCYGHRVFTKYPEEIPDYFKQAFPEGLSWERSLEFEDGGSASVSAHISLRGNTFYHKSKFTGVNFPADGPIMQNQSVDWEPSTEKITASDGVLKGDVTMYLKLEGGGNHKCQFKTTYKAAKEILEMPGDHYIGHRLVRKTEGNITEQVEDAVAHSMKTVKVNITTPDGPVYDADIEMVSVRAESGDLGILPGHIPTKAPLKIGAVRLKKDGQTEMVAVSGGTVEVRPDHVTINAQAAETAEGIDKERAEAARQRAQERLNSQSDDTDIRRAELALQRALNRLDVAGKFFDGSVQLADHYQQNTPIGDGPVLLPDNHYLSTQSKLSKDPNEKRDHMVLLEFVTAAGITLGMDELYKGGSGGMVSKGEELFTGVVPILVELDGDVNGHKFSVSGEGEGDATYGKLTLKFICTTGKLPVPWPTLVTTLTYGVQCFSRYPDHMKQHDFFKSAMPEGYVQERTIFFKDDGNYKTRAEVKFEGDTLVNRIELKGIDFKEDGNILGHKLEYNYNSHNVYIMADKQKNGIKVNFKIRHNIEEA

SEQ ID NO: 10 - protein, 599 aa, Artificial Sequence
  Synthetic
  MISC_FEATURE (1)..(1): optionally absent
  MISC_FEATURE (220)..(220): optionally absent
MVSVIKPEMKMRYYMDGSVNGHEFTIEGEGTGRPYEGHQEMTLRVTMAEGGPMPFAFDLVSHVFCYGHRVFTKYPEEIPDYFKQAFPEGLSWERSLEFEDGGSASVSAHISLRGNTFYHKSKFTGVNFPADGPIMQNQSVDWEPSTEKITASDGVLKGDVTMYLKLEGGGNHKCQFKTTYKAAKEILEMPGDHYIGHRLVRKTEGNITEQVEDAVAHSVMKTVKVNITTPDGPVYDADIEMVSVRAESGDLGILPGHIPTKAPLKIGAVRLKKDGQTEMVAVSGGTVEVRPDHVTINAQAAETAEGIDKERAEAARQRAQERLNSQSDDTDIRRAELALQRALNRLDVAGKFLDGSVQLADHYQQNTPIGDGPVLLPDNHYLSTQSKLSKDPNEKRDHMVLLEFVTAAGITLGMDELYKGGSGGMVSKGEELFTGVVPILVELDGDVNGHKFSVSGEGEGDATYGKLTLKFICTTGKLPVPWPTLVTTLTYGVQCFSRYPDHMKQHDFFKSAMPEGYVQERTIFFKDDGNYKTRAEVKFEGDTLVNRIELKGIDFKEDGNILGHKLEYNYNSHNVYIMADKQKNGIKVNFKIRHNIEEA

SEQ ID NO: 11 - protein, 601 aa, Artificial Sequence
  Synthetic
  MISC_FEATURE (1)..(1): optionally absent
  MISC_FEATURE (220)..(220): optionally absent
MVSVIKPEMKMRYYMDGSVNGHEFTIEGEGTGRPYEGHQEMTLRVTMAEGGPMPFAFDLVSHVFCYGHRVFTKYPEEIPDYFKQAFPEGLSWERSLEFEDGGSASVSAHISLRGNTFYHKSKFTGVNFPADGPIMQNQSVDWEPSTEKITASDGVLKGDVTMYLKLEGGGNHKCQFKTTYKAAKEILEMPGDHYIGHRLVRKTEGNITEQVEDAVAHSTMKTVKVNITTPDGPVYDADIEMVSVRAESGDLGILPGHIPTKAPLKIGAVRLKKDGQTEMVAVSGGTVEVRPDHVTINAQAAETAEGIDKERAEAARQRAQERLNSQSDDTDIRRAELALQRALNRLDVAGKGTSGDGSVQLADHYQQNTPIGDGPVLLPDNHYLSTQSKLSKDPNEKRDHMVLLEFVTAAGITLGMDELYKGGSGGMVSKGEELFTGVVPILVELDGDVNGHKFSVSGEGEGDATYGKLTLKFICTTGKLPVPWPTLVTTLTYGVQCFSRYPDHMKQHDFFKSAMPEGYVQERTIFFKDDGNYKTRAEVKFEGDTLVNRIELKGIDFKEDGNILGHKLEYNYNSHNVYIMADKQKNGIKVNFKIRHNIEEA

SEQ ID NO: 12 - protein, 132 aa, Artificial Sequence
  Synthetic
  MISC_FEATURE (1)..(1): optionally absent
MKTVKVNITTPDGPVYDADIEMVSVRAESGDLGILPGHIPTKAPLKIGAVRLKKDGQTEMVAVSGGTVEVRPDHVTINAQAAETAEGIDKERAEAARQRAQERLNSQSDDTDIRRAELALQKALNKLDVAGK

SEQ ID NO: 13 - protein, 598 aa, Artificial Sequence
  Synthetic
MVSVIKPEMKMRYYMDGSVNGHEFTIEGEGTGRPYEGHQEMTLRVTMAEGGPMPFAFDLVSHVFCYGHRVFTKYPEEIPDYFKQAFPEGLSWERSLEFEDGGSASVSAHISLRGNTFYHKSKFTGVNFPADGPIMQNQSVDWEPSTEKITASDGVLKGDVTMYLKLEGGGNHKCQFKTTYKAAKEILEMPGDHYIGHRLVRKTEGNITEQVEDAVAHSAMKTVKVNITTPDGPVYDADIEMVSVRAESGDLGILPGHIPTKAPLKIGAVRLKKDGQTEMVAVSGGTVEVRPDHVTINAQAAETAEGIDKERAEAARQRAQERLNSQSDDTDIRRAELALQKALNKLDVAGKADGSVQLADHYQQNTPIGDGPVLLPDNHYLSTQSKLSKDPNEKRDHMVLLEFVTAAGITLGMDELYKGGSGGMVSKGEELFTGVVPILVELDGDVNGHKFSVSGEGEGDATYGKLTLKFICTTGKLPVPWPTLVTTLTYGVQCFSRYPDHMKQHDFFKSAMPEGYVQERTIFFKDDGNYKTRAEVKFEGDTLVNRIELKGIDFKEDGNILGHKLEYNYNSHNVYIMADKQKNGIKVNFKIRHNIEEA

SEQ ID NO: 14 - DNA, 396 bp, Artificial Sequence
  Synthetic
atgaaaactgtgaaagtgaatataacaacccctgatgggccagtctacgacgctgatatcgagatggtgtccgtgcgggccgagagtggtgatctcggcatcctccccggtcacattcccacaaaggccccactgaagatcggagctgtgcggctgaagaaggacggccaaaccgagatggtcgcagtctcaggcggcactgttgaagtgcggcctgaccacgttaccattaatgctcaagccgctgaaacagccgaaggaatcgacaaagagagagcagaagccgcaagacagagggcccaggagcggctgaactctcaatccgatgacaccgatattcgccgggccgagctggcactgcagagggccctgaacagactggacgtggctgggaag

SEQ ID NO: 15 - protein, 132 aa, Artificial Sequence; identical to SEQ ID NO: 12
  Synthetic

SEQ ID NO: 16 - DNA, 396 bp, Artificial Sequence
  Synthetic
atgaaaactgtgaaagtgaatataacaacccctgatgggccagtctacgacgctgatatcgagatggtgtccgtgcgggccgagagtggtgatctcggcatcctccccggtcacattcccacaaaggccccactgaagatcggagctgtgcggctgaagaaggacggccaaaccgagatggtcgcagtctcaggcggcactgttgaagtgcggcctgaccacgttaccattaatgctcaagccgctgaaacagccgaaggaatcgacaaagagagagcagaagccgcaagacagagggcccaggagcggctgaactctcaatccgatgacaccgatattcgccgggccgagctggcactgcagaaggccctgaacaagctggacgtggctgggaag

SEQ ID NO: 17 - DNA, 1794 bp, Artificial Sequence
  Synthetic
atggtgagtgtgattaaaccagagatgaagatgaggtactacatggacggctccgtcaatgggcatgagttcacaattgaaggtgaaggcacaggcagaccttacgagggacatcaagagatgacactacgcgtcacaatggccgagggcgggccaatgcctttcgcgtttgacttagtgtcacacgtgttctgttacggccacagagtatttactaaatatccagaagagataccagactatttcaaacaagcatttcctgaaggcctgtcatgggaaaggtcgttggagttcgaagatggtgggtccgcttcagtcagtgcgcatataagccttagaggaaacaccttctaccacaaatccaaatttactggggttaactttcctgccgatggtcctatcatgcaaaaccaaagtgttgattgggagccatcaaccgagaaaattactgccagcgacggagttctgaagggtgatgttacgatgtacctaaaacttgaaggaggcggcaatcacaaatgccaattcaagactacttacaaggcggcaaaagagattcttgaaatgccaggagaccattacatcggccatcgcctcgtcaggaaaaccgaaggcaacattactgagcaggtagaagatgcagtagctcattccgctatgaaaactgtgaaagtgaatataacaacccctgatgggccagtctacgacgctgatatcgagatggtgtccgtgcgggccgagagtggtgatctcggcatcctccccggtcacattcccacaaaggccccactgaagatcggagctgtgcggctgaagaaggacggccaaaccgagatggtcgcagtctcaggcggcactgttgaagtgcggcctgaccacgttaccattaatgctcaagccgctgaaacagccgaaggaatcgacaaagagagagcagaagccgcaagacagagggcccaggagcggctgaactctcaatccgatgacaccgatattcgccgggccgagctggcactgcagagggccctgaacagactggacgtggctgggaaggctgacggcagcgtgcagctcgccgaccactaccagcagaacacccccatcggcgacggccccgtgctgctgcccgacaaccactacctgagcacccagtccaagctgagcaaagaccccaacgagaagcgcgatcacatggtcctgctggagttcgtgaccgccgccgggatcactctcggcatggacgagctgtacaagggtggcagcggtggcatggtgagcaagggcgaggagctgttcaccggggtggtgcccatcctggtcgagctggacggcgacgtaaacggccacaagttcagcgtgtccggcgagggcgagggcgatgccacctacggcaagctgaccctgaagttcatctgcaccaccggcaagctgcccgtgccctggcccaccctcgtgaccaccctgacctacggcgtgcagtgcttcagccgctaccccgaccacatgaagcagcacgacttcttcaagtccgccatgcccgaaggctacgtccaggagcgcaccatcttcttcaaggacgacggcaactacaagacccgcgccgaggtgaagttcgagggcgacaccctggtgaaccgcatcgagctgaagggcatcgacttcaaggaggacggcaacatcctggggcacaagctggagtacaactacaacagccacaacgtctatatcatggccgacaagcagaagaacggcatcaaggtgaacttcaagatccgccacaacatcgaggaagct

SEQ ID NO: 18 - DNA, 1794 bp, Artificial Sequence
  Synthetic
atggtgagtgtgattaaaccagagatgaagatgaggtactacatggacggctccgtcaatgggcatgagttcacaattgaaggtgaaggcacaggcagaccttacgagggacatcaagagatgacactacgcgtcacaatggccgagggcgggccaatgcctttcgcgtttgacttagtgtcacacgtgttctgttacggccacagagtatttactaaatatccagaagagataccagactatttcaaacaagcatttcctgaaggcctgtcatgggaaaggtcgttggagttcgaagatggtgggtccgcttcagtcagtgcgcatataagccttagaggaaacaccttctaccacaaatccaaatttactggggttaactttcctgccgatggtcctatcatgcaaaaccaaagtgttgattgggagccatcaaccgagaaaattactgccagcgacggagttctgaagggtgatgttacgatgtacctaaaacttgaaggaggcggcaatcacaaatgccaattcaagactacttacaaggcggcaaaagagattcttgaaatgccaggagaccattacatcggccatcgcctcgtcaggaaaaccgaaggcaacattactgagcaggtagaagatgcagtagctcattccgctatgaaaactgtgaaagtgaatataacaacccctgatgggccagtctacgacgctgatatcgagatggtgtccgtgcgggccgagagtggtgatctcggcatcctccccggtcacattcccacaaaggccccactgaagatcggagctgtgcggctgaagaaggacggccaaaccgagatggtcgcagtctcaggcggcactgttgaagtgcggcctgaccacgttaccattaatgctcaagccgctgaaacagccgaaggaatcgacaaagagagagcagaagccgcaagacagagggcccaggagcggctgaactctcaatccgatgacaccgatattcgccgggccgagctggcactgcagaaggccctgaacaagctggacgtggctgggaaggctgacggcagcgtgcagctcgccgaccactaccagcagaacacccccatcggcgacggccccgtgctgctgcccgacaaccactacctgagcacccagtccaagctgagcaaagaccccaacgagaagcgcgatcacatggtcctgctggagttcgtgaccgccgccgggatcactctcggcatggacgagctgtacaagggtggcagcggtggcatggtgagcaagggcgaggagctgttcaccggggtggtgcccatcctggtcgagctggacggcgacgtaaacggccacaagttcagcgtgtccggcgagggcgagggcgatgccacctacggcaagctgaccctgaagttcatctgcaccaccggcaagctgcccgtgccctggcccaccctcgtgaccaccctgacctacggcgtgcagtgcttcagccgctaccccgaccacatgaagcagcacgacttcttcaagtccgccatgcccgaaggctacgtccaggagcgcaccatcttcttcaaggacgacggcaactacaagacccgcgccgaggtgaagttcgagggcgacaccctggtgaaccgcatcgagctgaagggcatcgacttcaaggaggacggcaacatcctggggcacaagctggagtacaactacaacagccacaacgtctatatcatggccgacaagcagaagaacggcatcaaggtgaacttcaagatccgccacaacatcgaggaagct

SEQ ID NO: 19 - protein, 598 aa, Artificial Sequence; identical to SEQ ID NO: 13
  Synthetic

SEQ ID NO: 20 - protein, 4 aa, Artificial Sequence
  Synthetic
PPPP

SEQ ID NO: 21 - protein, 4 aa, Artificial Sequence
  Synthetic
GTSG

SEQ ID NO: 22 - protein, 5 aa, Artificial Sequence
  Synthetic
ANEFM